European Patent Specification EP 3 274 451 B1, published January 1, 2025. Title: FRUCTOSE TO ALLULOSE CONVERSION. Applicant: ARCHER DANIELS MIDLAND CO. The sequence listing filed with the application follows.

SEQUENCE LISTING (26 sequences)

SEQ ID NO: 1 - protein, 290 aa, Burkholderia RPE64
MNKVGMFYTYWSTEWLVDFPAVAKRISGLGFDMMEISLSEFHNLPDAKKRELKTVADDLGLTVMCCIGLKPEYDFASPEQSVRDAGTEYVKHLLDDCHMLGAPVFAGLTFCAWPQSPPPGMKDKRPYVERAVDSVRRVIKVAEGYGIIYALEVVNRFEQWLANDAREALAFCDAVDNPWCKVQLDTFHMNIEENSFRDAILACRGRLGHFHLGEANRLPPGEGRLPWDEIFGALKEIDYDGTIVMEPFMRPGGSVSRAVGVWRDMSNGATDEQMDERARRSLNFVRGHLA

SEQ ID NO: 2 - DNA, 870 bp, Burkholderia RPE64
atgaacaaagtaggcatgttctatacatactggtcgactgaatggctcgtggattttccggctgtggcgaagcgcatctcgggtctgggtttcgacatgatggagatctcgctctccgagttccataacttgcctgatgcgaagaagcgcgaactcaagaccgtcgccgacgatctcggtttgacggtgatgtgctgcatcggtctcaagcctgagtacgatttcgcatcgccggaacagagcgtgcgcgatgcgggcacggaatacgtgaagcatctgctcgacgattgccacatgctcggcgcaccggttttcgcgggcctgacattctgcgcgtggccgcaatcgccgccgccaggcatgaaggacaagcgtccatacgtcgaacgcgcggtggacagcgtgcgccgtgtcatcaaggtcgctgaaggttacggcattatctacgcgctggaagtggtgaatcgcttcgagcaatggctcgccaacgatgcacgcgaggcgctcgcgttctgcgatgcagtcgataatccgtggtgcaaggtgcagctcgatacgttccacatgaacatcgaagagaactcgtttcgcgatgccattctcgcgtgccgcggccgtctcggacacttccatctcggcgaagcgaaccgcttgccgccgggcgaaggccgtctgccgtgggatgaaatcttcggcgcgttgaaagagatcgactacgacggcaccatcgtcatggagccgttcatgcgtcctggcggctcggtgagtcgtgccgtgggcgtctggcgcgacatgtcgaacggcgcgacggatgaacagatggacgaacgcgcacgccgttcattgaacttcgtgcgcggtcatctcgcg

SEQ ID NO: 3 - DNA, 25 bp, Artificial Sequence
  PCR Primer
ggaattgtgagcggataacaattcc

SEQ ID NO: 4 - DNA, 38 bp, Artificial Sequence
  PCR Primer
attgctcgagttacgcgagatgaccgcgcacgaagttc

SEQ ID NO: 5 - DNA, 38 bp, Artificial Sequence
  PCR Primer
gaatcccacgtagtgcggctggatacggcgggcgcacg

SEQ ID NO: 6 - DNA, 38 bp, Artificial Sequence
  PCR Primer
gctaatttaaattactgatgattcatcatcaatttacg

SEQ ID NO: 7 - DNA, 2653 bp, Artificial Sequence
  gene cassette that was used to create ASR182
cgcggcaggcggtcgcggaaatcggcgcggtagcgagcggtatctccggctccggcccgaccttgttcgctctgtgtgacaagccggaaaccgcccagcgcgttgccgactggttgggtaagaactacctgcaaaatcaggaaggttttgttcatatttgccggctggatacggcgggcgcacgagtactggaaaactaaatgaaactctacaatctgaaagatcacaacgagcaggtcagctttgcgcaagccgtaacccaggggttgggcaaaaatcaggggctgttttttccgcacgacctgccggaattcagcctgactgaaattgatgagatgctgaagctggattttgtcacccgcagtgcgaagatcctctcggcgtttattggtgatgaaatcccacaggaaatcctggaagagcgcgtgcgcgcggcgtttgccttcccggctccggtcgccaatgttgaaagcgatgtcggttgtctggaattgttccacgggccaacgctggcatttaaagatttcggcggtcgctttatggcacaaatgctgacccatattgcgggtgataagccagtgaccattctgaccgcgacctccggtgataccggagcggcagtggctcatgctttctacggtttaccgaatgtgaaagtggttatcctctatccacgaggcaaaatcagtccactgcaagaaaaactgttctgtacattgggcggcaatatcgaaactgttgccatcgacggcgatttcgatgcctgtcaggcgctggtgaagcaggcgtttgatgatgaagaactgaaagtggcgctagggttaaactcggctaactcgattaacatcagccgtttgctggcgcagatttgctactactttgaagctgttgcgcagctgccgcaggagacgcgcaaccagctggttgtctcggtgccaagcggaaacttcggcgatttgacggcgggtctgctggcgaagtcactcggtctgccggtgaaacgttttattgctgcgaccaacgtgaacgataccgtgccacgtttcctgcacgacggtcagtggtcacccaaagcgactcaggcgacgttatccaacgcgatggacgtgagtcagccgaacaactggccgcgtgtggaagagttgttccgccgcaaaatctggcaactgaaagagctgggttatgcagccgtggatgatgaaaccacgcaacagacaatgcgtgagttaaaagaactgggctacacttcggagccgcacgctgccgtagcttatcgtgcgctgcgtgatcagttgaatccaggcgaatatggcttgttcctcggcaccgcgcatccggcgaaatttaaagagagcgtggaagcgattctcggtgaaacgttggatctgccaaaagagctggcagaacgtgctgatttacccttgctttcacataatctgcccgccgattttgctgcgttgcgtaaattgatgatgaatcatcagtaagaaattaatacgactcactataggggaattgtgagcggataacaattcccctctagaaataattttgtttaactttaagaaggagatatacatatgaacaaagtaggcatgttctatacatactggtcgactgaatggctcgtggattttccggctgtggcgaagcgcatctcgggtctgggtttcgacatgatggagatctcgctctccgagttccataacttgcctgatgcgaagaagcgcgaactcaagaccgtcgccgacgatctcggtttgacggtgatgtgctgcatcggtctcaagcctgagtacgatttcgcatcgccggaacagagcgtgcgcgatgcgggcacggaatacgtgaagcatctgctcgacgattgccacatgctcggcgcaccggttttcgcgggcctgacattctgcgcgtggccgcaatcgccgccgccaggcatgaaggacaagcgtccatacgtcgaacgcgcggtggacagcgtgcgccgtgtcatcaaggtcgctgaaggttacggcattatctacgcgctggaagtggtgaatcgcttcgagcaatggctcgccaacgatgcacgcgaggcgctcgcgttctgcgatgcagtcgataatccgtggtgcaaggtgcagctcgatacgttccacatgaacatcgaagagaactcgtttcgcgatgccattctcgcgtgccgcggccgtctcggacacttccatctcggcgaagcgaaccgcttgccgccgggcgaaggccgtctgccgtgggatgaaatcttcggcgcgttgaaagagatcgactacgacggcaccatcgtcatggagccgttcatgcgtcctggcggctcggtgagtcgtgccgtgggcgtctggcgcgacatgtcgaacggcgcgacggatgaacagatggacgaacgcgcacgccgttcattgaacttcgtgcgcggtcatctcgcgtaaaatctattcattatctcaatcaggccgggtttgcttttatgcagcccggcttttttatgaagaaattatggagaaaaatgacagggaaaaaggagaaattctcaataaatgcggtaacttagagattaggattgcggagaataacaaccgccgttctcatcgagtaatctccggatatcgacccataacgggcaatgata

SEQ ID NO: 8 - DNA, 26 bp, Artificial Sequence
  PCR Primer
cgcggcaggcggtcgcggaaatcggc

SEQ ID NO: 9 - DNA, 27 bp, Artificial Sequence
  PCR Primer
tatcattgcccgttatgggtcgatatc

SEQ ID NO: 10 - DNA, 879 bp, Artificial Sequence
  nucleotide sequence that encodes the polypeptide sequence of SEQ ID NO: 1 with an NdeI and XhoI
catatgaacaaagtaggcatgttctatacatactggtcgactgaatggctcgtggattttccggctgtggcgaagcgcatctcgggactgggtttcgacatgatggagatatcgctctccgagttccataacttgcccgatgcgaagaagcgcgaactaaagaccgtcgccgacgatctcggtttgacggtgatgtgctgcatcggtctcaagcccgagtacgatttcgcatcgccggaacagagcgtgcgcgatgcgggcacggaatacgtgaagcatctgctcgacgattgccatatgctcggcgcaccggttttcgcgggcctgacattctgcgcgtggccgcaatcgccgccgcccggcatgaaggacaagcgtccatacgtcgaacgcgcggtggacagcgtgcggcgtgtcatcaaggtcgctgaagggtacggcattatctacgcgctggaagtggtgaatcgcttcgagcaatggctcgccaacgatgcacgcgaggcgctcgcgttctgcgatgcagtcgataatccgtggtgcaaggtgcagctcgatacgttccacatgaacatcgaagagaactcgtttcgcgatgccattctcgcgtgccgcggcaggctcggacacttccatctcggcgaagcgaaccgcttgccgccgggcgaaggccgtctgccgtgggatgaaatcttcggcgcgttgaaagagatcgactacgacggcaccatcgtcatggagccgttcatgcgtccgggcggctcggtgagtcgtgccgtgggcgtctggcgcgacatgtcgaacggcgcgacggatgaacagatggacgaacgcgcacgccgctcattgaacttcgtgcgcggacatctcgcgctcgag

SEQ ID NO: 11 - protein, 300 aa, Pseudomonas cichorii
MNKVGMFYTYWSTEWMVDFPATAKRIAGLGFDLMEISLGEFHNLSDAKKRELKAVADDLGLTVMCSIGLKSEYDFASPDKSVRDAGTEYVKRLLDDCHLLGAPVFAGLTFCAWPQSPPLDMKDKRPYVDRAIESVRRVIKVAEDYGIIYALEVVNRFEQWLCNDAKEAIAFADAVDSPACKVQLDTFHMNIEETSFRDAILACKGKMGHFHLGEANRLPPGEGRLPWDEIFGALKEIGYDGTIVMEPFMRKGGSVSRAVGVWRDMSNGATDEEMDERARRSLQFVRDKLAGSRSHHHHHH

SEQ ID NO: 12 - protein, 289 aa, Candidatus Burkholderia verscheurenii
MNKVGMFYTYWSTEWLVDFPAVAKRISELGFDMMEISLSEFHTLPDAKKRELKAVADDLGLTVMCCIGLKQEYDFASPEQSVRDAGTEYVKRLLDDCHMLGAPVFAGLTFCAWPQSPPPGMKDKRPYVERAIDSVRRVIKVAEGYVIYALEIVNRFEQWLANDAREALAFCDAVDNPWCRVQLDTFHMNIEENSFRDAILACKWRLGHFHLGEANRLPPGEGRLPWDEIFGALKEIDYDGTIVMEPFMRPGGSVSRAVGVWHDMSNGATDEQMDERARRSLQFVRGRLS

SEQ ID NO: 13 - protein, 290 aa, Burkholderia jiangsuensis
MNKVGMFYTYWSTEWMVDFPATAKRIAGLGFDMMEISLGEFHNLPDAKKRELKAIADDLGLTVMCCIGLKPEYDFASPEQSVRDAGTEYVKRLLDDCHMLGAPVFAGLTFCAWPQSPPPGMKDKRPYVDHAIDSVRRVIKVAEDYGIIYALEVVNRFEQWLCNDAKEALAFVDAVDSPACKVQLDTFHMNIEEHSFRDAILACKGKLGHFHLGEANRLPPGEGRLPWDEIFGALKEIGYDGTIVMEPFMRKGGSVSRAVGVWRDMSNGATDEQMDERARRSLQFVRGKLT

SEQ ID NO: 14 - protein, 290 aa, Burkholderia sp.
MNKVGMFYTYWSTEWMVDFPATAKRIAGLGFDMMEISLGEFHNLSDAKKRELKTVADDLGLTVMCCIGLKSEYDFASPEQSVRDAGTEYVKRLLDDCHMLGAPVFAGLTFCAWPQSPPLDMKDKRPYVDRAIDSVRRVVKVAEDYGIIYALEVVNRFEQWLCNDAKEALAFADAVDSPACKVQLDTFHMNIEESSFRDAILACKGKLGHFHLGEANRLPPGEGRLPWDEIFGALKEIDYDGTIVMEPFMRKGGAVSRAVGVWRDMSNGATDEQMDERARRSLQFVRGKLA

SEQ ID NO: 15 - protein, 291 aa, Burkholderia sp.
MNKVGMFYTYWSTEWMVDFPATARRIAGLGFDMMEISLGEFHNLPDAKKRELKTVADDLGLTVMCCIGLKPEYDFASPEQSVRDAGTEYVKRLLDDCHMLNAPVFAGLTFCAWPQSPPLDMKDKRPYVDRAIDSVRRVIDVAEGYGIIYALEVVNRFEQWLCNDAKEAIAFADAVGSPACKVQLDTFHMNIEESSFRDAILACKGKLGHFHLGEANRLPPGEGRLPWDEIFGALKEIDYDGTIVMEPFMRKGGPVSRAVGVWRDMSNGATDEQMDERARRSLQFVRGKLSS

SEQ ID NO: 16 - protein, 290 aa, Burkholderia sp. MR1
MNKVGMFYTYWSTEWMVDFPATAKRIAGLGFDMMEISLGEFHNLPDAKKRELKSVADDLGLTVMCCIGLKSEYDFASPDKSVRDAGTEYVKRLLDDCHLLGAPVFAGLTFCAWPQSPPLDMKDKRPYVDRAIDSVRRVIKVAEDYGIIYALEVVNRFEQWLCNDAKEALAFADAVDSPACKVQLDTFHMNIEESSFRDAILACKGKMGHFHLGEANRLPPGEGRLPWDEIFGALKEIEYDGTIVMEPFMRKGGSVSRAVGVWRDMSNGATDEQMDERARRSLQFVREKLA

SEQ ID NO: 17 - protein, 285 aa, Burkholderia jiangsuensis
MFYTYWSTEWMVDFPATAKRIAGLGFDMMEISLGEFHNLPDAKKRELKAIADDLGLTVMCCIGLKPEYDFASPEQSVRDAGTEYVKRLLDDCHMLGAPVFAGLTFCAWPQSPPPGMKDKRPYVDHAIDSVRRVIKVAEDYGIIYALEVVNRFEQWLCNDAKEALAFVDAVDSPACKVQLDTFHMNIEEHSFRDAILACKGKLGHFHLGEANRLPPGEGRLPWDEIFGALKEIGYDGTIVMEPFMRKGGSVSRAVGVWRDMSNGATDEQMDERARRSLQFVRGKLT

SEQ ID NO: 18 - protein, 290 aa, Burkholderia grimmiae
MNKVGMFYTYWSTEWMVDFPATAKRIAGLGFDLMEISLGEFHNLPDAKKRELKAVADDLGLTVMCCIGLKSEYDFASPDKSVRDAGTEYVKRLLDDCHLLGAPVFAGLTFCAWPQSPPLDMRDKRPYVDRAIEGVRRVIKVAEDYGIIYALEVVNRFEQWLCNDAKEAIAFADAVDSPACKVQLDTFHMNIEETSFRDAILACKGKMGHFHLGEANRLPPGEGRLPWDEIFGALKEIGYDGTIVMEPFMRKGGSVSRAVGVWRDMSNGATDEEMDERARRSLQFVRDKLA

SEQ ID NO: 19 - protein, 298 aa, Burkholderia sp.
MNKVGMFYTYWSTEWMVDFPATAKRIAGLGFDLMEISLGEFHNLSDAKKRELKAVADDLGLTVMCCIGLKSEYDFASPDKSVRDAGTEYVKRLLDDCHLLGAPVFAGLTFCAWPQHPPLDMVDKRPYVDRAIESVRRVIKVAEDYGIIYALEVVNRYEQWLCNDAKEAIAFADAVDSPACKVQLDTFHMNIEENSFRDAILACKGKMGHFHLGEQNRLPPGEGRLPWDEIFGALKEIGYDGTIVMEPFMRTGGSVSRAVCVWRDLSNGATDEEMDERARRSLQFVRDKLALEHHHHHH

SEQ ID NO: 20 - protein, 285 aa, Burkholderia grimmiae
MFYTYWSTEWMVDFPATAKRIAGLGFDLMEISLGEFHNLPDAKKRELKAVADDLGLTVMCCIGLKSEYDFASPDKSVRDAGTEYVKRLLDDCHLLGAPVFAGLTFCAWPQSPPLDMRDKRPYVDRAIEGVRRVIKVAEDYGIIYALEVVNRFEQWLCNDAKEAIAFADAVDSPACKVQLDTFHMNIEETSFRDAILACKGKMGHFHLGEANRLPPGEGRLPWDEIFGALKEIGYDGTIVMEPFMRKGGSVSRAVGVWRDMSNGATDEEMDERARRSLQFVRDKLA

SEQ ID NO: 21 - protein, 298 aa, Burkholderia sp.
MNKVGMFYSYWSTEWMVDFPATAKRIAGLGFDLMEISLSEFHNLSDAKKRELKAVADDLGLTVMCCIGLKSEYDFASPDKSVRDAGTEYVKRLLDDCHLLGAPVFAGLNFCAWPQHPPLDMVDKRPYVDRAIESVRRVIKVAEDYGIIYALEAVNRYEQWLCNDAKEAIAFADAVDSPACKVHLDTFHMNIEENSFRDAILACKGKMGHFHLGEQNRLPPGEGRLPWDEIFGALKEIGYDGTIVIEPFMRTGGSVSRAVCVWRDLSNGATDEEMDERARRSLQFVRDKLALEHHHHHH

SEQ ID NO: 22 - protein, 298 aa, Burkholderia sp.
MNKVGMFYTYWSTEWMVDFPATAKRIAGLGFDLMEINLEEFHNLSDAKKRELKAVADDLGLTVMCCIGLKSEYDFASPDKSVRDAGTEYVKRLLDDCHLLGAPVFAGLNFCAWPQHPPLDMVDKRPYVDRAIESVRRVIKVAEDYGIIYALEVVNRYEQWLCNDAKEAIAFADAVDSPACKVQLDTFHMNIEENSFRDAILACKGKMGVFHIGEQNRLPPGEGRLPWDEIFGALKEIGYDGTIVMEPFMRTGGSVGRDVCVWRDLSNGATDEEMDERARRSLQFVRDKLALEHHHHHH

SEQ ID NO: 23 - protein, 275 aa, Burkholderia sp. MR1
MVDFPATAKRIAGLGFDMMEISLGEFHNLPDAKKRELKSVADDLGLTVMCCIGLKSEYDFASPDKSVRDAGTEYVKRLLDDCHLLGAPVFAGLTFCAWPQSPPLDMKDKRPYVDRAIDSVRRVIKVAEDYGIIYALEVVNRFEQWLCNDAKEALAFADAVDSPACKVQLDTFHMNIEESSFRDAILACKGKMGHFHLGEANRLPPGEGRLPWDEIFGALKEIEYDGTIVMEPFMRKGGSVSRAVGVWRDMSNGATDEQMDERARRSLQFVREKLA

SEQ ID NO: 24 - protein, 158 aa, Candidatus Burkholderia brachyanthoides
MMEISLSEFHTLPETKKRELKTVADDLGLTVMCCIGLKQEYDFASPEQSVRDAGTEYVKRLLDDCHMLGAPVFAGRTFCAWPQSPPPGMTDKRPYVDRAIDSVRRMIKVAEGHGIIYALEVVNRFQQWLANDAREALAFCDAVDNPWCRVQFVRGHLA

SEQ ID NO: 25 - protein, 157 aa, Candidatus Burkholderia brachyanthoides
MEISLSEFHTLPETKKRELKTVADDLGLTVMCCIGLKQEYDFASPEQSVRDAGTEYVKRLLDDCHMLGAPVFAGRTFCAWPQSPPPGMTDKRPYVDRAIDSVRRMIKVAEGHGIIYALEVVNRFQQWLANDAREALAFCDAVDNPWCRVQFVRGHLA

SEQ ID NO: 26 - protein, 138 aa, Candidatus Burkholderia calva
MVKRFEQWLANDAREALAFCDAVDNSWCRVQLDTFHMNIEENSFRDAILACKGRLGHFHLGEANCLPPGEGRLPWDEIFGALKEIGYDGTIVMEPFMRKGGSVSRAMGVWRDMSNGASDEQMDERARKSLQFARGHLA